European Patent Application EP 4 180 524 A1, published May 17, 2023. Title: 经修饰的谷氨酸脱氢酶及其应用. Applicant: 四川利尔生物科技有限公司. The sequence listing filed with the application follows.

SEQUENCE LISTING (72 sequences)

SEQ ID NO: 1 - protein, 457 aa, Bacillus vedderi
MTTTTVSNDQLAKEYVDGVFEQLKNQNSHQAEFLQAAEEIFISLVPVFAQHPEYIKANILSRIVEPDRIISFRVAWQDDNNQVQVNRGYRVQYSNVMGPYKGGLRFHPSVNESIIKFLGFEQIFKNALTGQPIGGGKGGSNFNPKGKSDSEIMRFCQAFMTELYRHIGPDVDVPAGDIGVGAREVGYLWGQYKRITKANESGVLTGKTPGYGGSLARKEATGYGTVYFVEEMLKEVNDSFEDKTVVVSGSGNVSTYAIEKAQAYGAKVVACSDSSGYIYDAEGLDLDVIKEIKEVKGDRISTYVDYRPNATFTEGCTGIWSIPCDIALPCATQNEINGDAARTLISNGVKAIGEGANMPSDLEAINEFLNAGVLFGPAKAANAGGVAVSALEMAQDSSRVFWTFEEVDAKLHQIMKNIYADSKAAADKYGYPGNLVVGANIAGFIKVADGMLAEGIY

SEQ ID NO: 2 - protein, 457 aa, Lysinibacillus sphaericus
MTITTVSNEQLAKEYVDGVFEQLKQQNCHQAEFLQAAEEIFISLVPVFVQHPEYIKANILSRIVEPDRIISFRVAWQDDHNQVQVNRGYRVQYSNVMGPYKGGLRFHPSVNESIIKFLGFEQIFKNALTGQPIGGGKGGSNFDPKGKSDSEIMRFCQAFMTELYRHIGPDVDVPAGDIGVGAREVGYLWGQYKRLTKASESGVLTGKTPGYGGSLARKEATGYGTVYFVNEMLKDVNDSFEGKTVVVSGSGNVSTYAIEKAQQYGAKVVACSDSSGYIYDPEGLDLDVIKEIKEVKGDRISTYVSYRPNATFTNGCTGIWTIPCDIALPCATQNEINGESARTLISNGVKAIGEGANMPSDLEAINEFLNAGVLFGPAKAANAGGVAVSALEMAQDSSRVFWSFEEVDAKLHQIMKDIYSDSKAAAEKYGFPGNLVMGANIAGFIKVADGMLTEGIY

SEQ ID NO: 3 - protein, 457 aa, Artificial Sequence
  mutant
MTTTTVSNDQLAKEYVDGVFEQLKNQNSHQAEFLQAAEEIFISLVPVFAQHPEYIKANILSRIVEPDRIISFRVAWQDDNNQVQVNRGYRVQYSNVMGPYKGGLRFHPSVNESIIKFLGFEQIFKNALTGQPIGGGKGGSNFNPKGKSDSEIMRFCQAFMTELYRHIGPDVDVPGGDIGVGAREVGYLWGQYKRITKANESGVLTGKTPGYGGSLARKEATGYGTVYFVEEMLKEVNDSFEDKTVVVSGSGNVSTYAIEKAQAYGAKVVACSDSSGYIYDAEGLDLDVIKEIKEVKGDRISTYVDYRPNATFTEGCTGIWSIPCDIALPCATQNEINGDAARTLISNGVKAIGEGANMPSDLEAINEFLNAGVLFGPAKAANAGGVAVSALEMAQDSSRVFWTFEEVDAKLHQIMKNIYADSKAAADKYGYPGNLVVGANIAGFIKVADGMLAEGIY

SEQ ID NO: 4 - protein, 457 aa, Artificial Sequence
  mutant
MTTTTVSNDQLAKEYVDGVFEQLKNQNSHQAEFLQAAEEIFISLVPVFAQHPEYIKANILSRIVEPDRIISFRVAWQDDNNQVQVNRGYRVQYSNVMGPYKGGCRFHPSVNESIIKFLGFEQIFKNALTGQPIGGGKGGSNFNPKGKSDSEIMRFCQAFMTELYRHIGPDVDVPGGDIGVGAREVGYLWGQYKRITKANESGVLTGKTPGYGGSLARKEATGYGTVYFVEEMLKEVNDSFEDKTVVVSGSGNVSTYAIEKAQAYGAKVVACSDSSGYIYDAEGLDLDVIKEIKEVKGDRISTYVDYRPNATFTEGCTGIWSIPCDIALPCATQNEINGDAARTLISNGVKAIGEGANMPSDLEAINEFLNAGVLFGPAKAANAGGVAVSALEMAQDSSRVFWTFEEVDAKLHQIMKNIYADSKAAADKYGYPGNLVVGANIAGFIKVADGMLAEGIY

SEQ ID NO: 5 - protein, 457 aa, Artificial Sequence
  mutant
MTTTTVSNDQLAKEYVDGVFEQLKNQNSHQAEFLQAAEEIFISLVPVFAQHPEYIKANILSRIVEPDRIISFRVAWQDDNNQVQVNRGYRVQYSNVMGPYKGGLRFHPSVNESIIKFLGFEQIFKNALTGQLIGGGKGGSNFNPKGKSDSEIMRFCQAFMTELYRHIGPDVDVPGGDIGVGAREVGYLWGQYKRITKANESGVLTGKTPGYGGSLARKEATGYGTVYFVEEMLKEVNDSFEDKTVVVSGSGNVSTYAIEKAQAYGAKVVACSDSSGYIYDAEGLDLDVIKEIKEVKGDRISTYVDYRPNATFTEGCTGIWSIPCDIALPCATQNEINGDAARTLISNGVKAIGEGANMPSDLEAINEFLNAGVLFGPAKAANAGGVAVSALEMAQDSSRVFWTFEEVDAKLHQIMKNIYADSKAAADKYGYPGNLVVGANIAGFIKVADGMLAEGIY

SEQ ID NO: 6 - protein, 457 aa, Artificial Sequence
  mutant
MTTTTVSNDQLAKEYVDGVFEQLKNQNSHQAEFLQAAEEIFISLVPVFAQHPEYIKANILSRIVEPDRIISFRVAWQDDNNQVQVNRGYRVQYSNVMGPYKGGLRFHPSVNESIIKFLGFEQIFKNALTGQPVGGGKGGSNFNPKGKSDSEIMRFCQAFMTELYRHIGPDVDVPGGDIGVGAREVGYLWGQYKRITKANESGVLTGKTPGYGGSLARKEATGYGTVYFVEEMLKEVNDSFEDKTVVVSGSGNVSTYAIEKAQAYGAKVVACSDSSGYIYDAEGLDLDVIKEIKEVKGDRISTYVDYRPNATFTEGCTGIWSIPCDIALPCATQNEINGDAARTLISNGVKAIGEGANMPSDLEAINEFLNAGVLFGPAKAANAGGVAVSALEMAQDSSRVFWTFEEVDAKLHQIMKNIYADSKAAADKYGYPGNLVVGANIAGFIKVADGMLAEGIY

SEQ ID NO: 7 - protein, 457 aa, Artificial Sequence
  mutant
MTTTTVSNDQLAKEYVDGVFEQLKNQNSHQAEFLQAAEEIFISLVPVFAQHPEYIKANILSRIVEPDRIISFRVAWQDDNNQVQVNRGYRVQYSNVMGPYKGGLRFHPSVNESIIKFLGFEQIFKNALTGQPIGGGKGGSNFNPKGKSDSEIMRFCQAFMTELYRHIGPDVDSPGGDIGVGAREVGYLWGQYKRITKANESGVLTGKTPGYGGSLARKEATGYGTVYFVEEMLKEVNDSFEDKTVVVSGSGNVSTYAIEKAQAYGAKVVACSDSSGYIYDAEGLDLDVIKEIKEVKGDRISTYVDYRPNATFTEGCTGIWSIPCDIALPCATQNEINGDAARTLISNGVKAIGEGANMPSDLEAINEFLNAGVLFGPAKAANAGGVAVSALEMAQDSSRVFWTFEEVDAKLHQIMKNIYADSKAAADKYGYPGNLVVGANIAGFIKVADGMLAEGIY

SEQ ID NO: 8 - protein, 457 aa, Artificial Sequence
  mutant
MTTTTVSNDQLAKEYVDGVFEQLKNQNSHQAEFLQAAEEIFISLVPVFAQHPEYIKANILSRIVEPDRIISFRVAWQDDNNQVQVNRGYRVQYSNVMGPYKGGLRFHPSVNESIIKFLGFEQIFKNALTGQPIGGGKGGSNFNPKGKSDSEIMRFCQAFMTELYRHIGPDVDGPGGDIGVGAREVGYLWGQYKRITKANESGVLTGKTPGYGGSLARKEATGYGTVYFVEEMLKEVNDSFEDKTVVVSGSGNVSTYAIEKAQAYGAKVVACSDSSGYIYDAEGLDLDVIKEIKEVKGDRISTYVDYRPNATFTEGCTGIWSIPCDIALPCATQNEINGDAARTLISNGVKAIGEGANMPSDLEAINEFLNAGVLFGPAKAANAGGVAVSALEMAQDSSRVFWTFEEVDAKLHQIMKNIYADSKAAADKYGYPGNLVVGANIAGFIKVADGMLAEGIY

SEQ ID NO: 9 - protein, 457 aa, Artificial Sequence
  mutant
MTTTTVSNDQLAKEYVDGVFEQLKNQNSHQAEFLQAAEEIFISLVPVFAQHPEYIKANILSRIVEPDRIISFRVAWQDDNNQVQVNRGYRVQYSNVMGPYKGGLRFHPSVNESIIKFLGFEQIFKNALTGQPIGGGKGGSNFNPKGKSDSEIMRFCQAFMTELYRHIGPDVDVPGGDIGVKAREVGYLWGQYKRITKANESGVLTGKTPGYGGSLARKEATGYGTVYFVEEMLKEVNDSFEDKTVVVSGSGNVSTYAIEKAQAYGAKVVACSDSSGYIYDAEGLDLDVIKEIKEVKGDRISTYVDYRPNATFTEGCTGIWSIPCDIALPCATQNEINGDAARTLISNGVKAIGEGANMPSDLEAINEFLNAGVLFGPAKAANAGGVAVSALEMAQDSSRVFWTFEEVDAKLHQIMKNIYADSKAAADKYGYPGNLVVGANIAGFIKVADGMLAEGIY

SEQ ID NO: 10 - protein, 457 aa, Artificial Sequence
  mutant
MTTTTVSNDQLAKEYVDGVFEQLKNQNSHQAEFLQAAEEIFISLVPVFAQHPEYIKANILSRIVEPDRIISFRVAWQDDNNQVQVNRGYRVQYSNVMGPYKGGLRFHPSVNESIIKFLGFEQIFKNALTGQPIGGGKGGSNFNPKGKSDSEIMRFCQAFMTELYRHIGPDVDVPGGDIGVRAREVGYLWGQYKRITKANESGVLTGKTPGYGGSLARKEATGYGTVYFVEEMLKEVNDSFEDKTVVVSGSGNVSTYAIEKAQAYGAKVVACSDSSGYIYDAEGLDLDVIKEIKEVKGDRISTYVDYRPNATFTEGCTGIWSIPCDIALPCATQNEINGDAARTLISNGVKAIGEGANMPSDLEAINEFLNAGVLFGPAKAANAGGVAVSALEMAQDSSRVFWTFEEVDAKLHQIMKNIYADSKAAADKYGYPGNLVVGANIAGFIKVADGMLAEGIY

SEQ ID NO: 11 - protein, 457 aa, Artificial Sequence
  mutant
MTTTTVSNDQLAKEYVDGVFEQLKNQNSHQAEFLQAAEEIFISLVPVFAQHPEYIKANILSRIVEPDRIISFRVAWQDDNNQVQVNRGYRVQYSNVMGPYKGGLRFHPSVNESIIKFLGFEQIFKNALTGQPIGGGKGGSNFNPKGKSDSEIMRFCQAFMTELYRHIGPDVDVPGGDIGVGRREVGYLWGQYKRITKANESGVLTGKTPGYGGSLARKEATGYGTVYFVEEMLKEVNDSFEDKTVVVSGSGNVSTYAIEKAQAYGAKVVACSDSSGYIYDAEGLDLDVIKEIKEVKGDRISTYVDYRPNATFTEGCTGIWSIPCDIALPCATQNEINGDAARTLISNGVKAIGEGANMPSDLEAINEFLNAGVLFGPAKAANAGGVAVSALEMAQDSSRVFWTFEEVDAKLHQIMKNIYADSKAAADKYGYPGNLVVGANIAGFIKVADGMLAEGIY

SEQ ID NO: 12 - protein, 457 aa, Artificial Sequence
  mutant
MTTTTVSNDQLAKEYVDGVFEQLKNQNSHQAEFLQAAEEIFISLVPVFAQHPEYIKANILSRIVEPDRIISFRVAWQDDNNQVQVNRGYRVQYSNVMGPYKGGLRFHPSVNESIIKFLGFEQIFKNALTGQPIGGGKGGSNFNPKGKSDSEIMRFCQAFMTELYRHIGPDVDVPGGDIGVGAREVGYLWGQYKRITKANESGILTGKTPGYGGSLARKEATGYGTVYFVEEMLKEVNDSFEDKTVVVSGSGNVSTYAIEKAQAYGAKVVACSDSSGYIYDAEGLDLDVIKEIKEVKGDRISTYVDYRPNATFTEGCTGIWSIPCDIALPCATQNEINGDAARTLISNGVKAIGEGANMPSDLEAINEFLNAGVLFGPAKAANAGGVAVSALEMAQDSSRVFWTFEEVDAKLHQIMKNIYADSKAAADKYGYPGNLVVGANIAGFIKVADGMLAEGIY

SEQ ID NO: 13 - protein, 457 aa, Artificial Sequence
  mutant
MTTTTVSNDQLAKEYVDGVFEQLKNQNSHQAEFLQAAEEIFISLVPVFAQHPEYIKANILSRIVEPDRIISFRVAWQDDNNQVQVNRGYRVQYSNVMGPYKGGLRFHPSVNESIIKFLGFEQIFKNALTGQLVGGGKGGSNFNPKGKSDSEIMRFCQAFMTELYRHIGPDVDVPGGDIGVGAREVGYLWGQYKRITKANESGVLTGKTPGYGGSLARKEATGYGTVYFVEEMLKEVNDSFEDKTVVVSGSGNVSTYAIEKAQAYGAKVVACSDSSGYIYDAEGLDLDVIKEIKEVKGDRISTYVDYRPNATFTEGCTGIWSIPCDIALPCATQNEINGDAARTLISNGVKAIGEGANMPSDLEAINEFLNAGVLFGPAKAANAGGVAVSALEMAQDSSRVFWTFEEVDAKLHQIMKNIYADSKAAADKYGYPGNLVVGANIAGFIKVADGMLAEGIY

SEQ ID NO: 14 - protein, 457 aa, Artificial Sequence
  mutant
MTTTTVSNDQLAKEYVDGVFEQLKNQNSHQAEFLQAAEEIFISLVPVFAQHPEYIKANILSRIVEPDRIISFRVAWQDDNNQVQVNRGYRVQYSNVMGPYKGGLRFHPSVNESIIKFLGFEQIFKNALTGQLIGGGKGGSNFNPKGKSDSEIMRFCQAFMTELYRHIGPDVDSPGGDIGVGAREVGYLWGQYKRITKANESGVLTGKTPGYGGSLARKEATGYGTVYFVEEMLKEVNDSFEDKTVVVSGSGNVSTYAIEKAQAYGAKVVACSDSSGYIYDAEGLDLDVIKEIKEVKGDRISTYVDYRPNATFTEGCTGIWSIPCDIALPCATQNEINGDAARTLISNGVKAIGEGANMPSDLEAINEFLNAGVLFGPAKAANAGGVAVSALEMAQDSSRVFWTFEEVDAKLHQIMKNIYADSKAAADKYGYPGNLVVGANIAGFIKVADGMLAEGIY

SEQ ID NO: 15 - protein, 457 aa, Artificial Sequence
  mutant
MTTTTVSNDQLAKEYVDGVFEQLKNQNSHQAEFLQAAEEIFISLVPVFAQHPEYIKANILSRIVEPDRIISFRVAWQDDNNQVQVNRGYRVQYSNVMGPYKGGLRFHPSVNESIIKFLGFEQIFKNALTGQLIGGGKGGSNFNPKGKSDSEIMRFCQAFMTELYRHIGPDVDGPGGDIGVGAREVGYLWGQYKRITKANESGVLTGKTPGYGGSLARKEATGYGTVYFVEEMLKEVNDSFEDKTVVVSGSGNVSTYAIEKAQAYGAKVVACSDSSGYIYDAEGLDLDVIKEIKEVKGDRISTYVDYRPNATFTEGCTGIWSIPCDIALPCATQNEINGDAARTLISNGVKAIGEGANMPSDLEAINEFLNAGVLFGPAKAANAGGVAVSALEMAQDSSRVFWTFEEVDAKLHQIMKNIYADSKAAADKYGYPGNLVVGANIAGFIKVADGMLAEGIY

SEQ ID NO: 16 - protein, 457 aa, Artificial Sequence
  mutant
MTTTTVSNDQLAKEYVDGVFEQLKNQNSHQAEFLQAAEEIFISLVPVFAQHPEYIKANILSRIVEPDRIISFRVAWQDDNNQVQVNRGYRVQYSNVMGPYKGGLRFHPSVNESIIKFLGFEQIFKNALTGQLIGGGKGGSNFNPKGKSDSEIMRFCQAFMTELYRHIGPDVDVPGGDIGVGRREVGYLWGQYKRITKANESGVLTGKTPGYGGSLARKEATGYGTVYFVEEMLKEVNDSFEDKTVVVSGSGNVSTYAIEKAQAYGAKVVACSDSSGYIYDAEGLDLDVIKEIKEVKGDRISTYVDYRPNATFTEGCTGIWSIPCDIALPCATQNEINGDAARTLISNGVKAIGEGANMPSDLEAINEFLNAGVLFGPAKAANAGGVAVSALEMAQDSSRVFWTFEEVDAKLHQIMKNIYADSKAAADKYGYPGNLVVGANIAGFIKVADGMLAEGIY

SEQ ID NO: 17 - protein, 457 aa, Artificial Sequence
  mutant
MTTTTVSNDQLAKEYVDGVFEQLKNQNSHQAEFLQAAEEIFISLVPVFAQHPEYIKANILSRIVEPDRIISFRVAWQDDNNQVQVNRGYRVQYSNVMGPYKGGLRFHPSVNESIIKFLGFEQIFKNALTGQPVGGGKGGSNFNPKGKSDSEIMRFCQAFMTELYRHIGPDVDSPGGDIGVGAREVGYLWGQYKRITKANESGVLTGKTPGYGGSLARKEATGYGTVYFVEEMLKEVNDSFEDKTVVVSGSGNVSTYAIEKAQAYGAKVVACSDSSGYIYDAEGLDLDVIKEIKEVKGDRISTYVDYRPNATFTEGCTGIWSIPCDIALPCATQNEINGDAARTLISNGVKAIGEGANMPSDLEAINEFLNAGVLFGPAKAANAGGVAVSALEMAQDSSRVFWTFEEVDAKLHQIMKNIYADSKAAADKYGYPGNLVVGANIAGFIKVADGMLAEGIY

SEQ ID NO: 18 - protein, 457 aa, Artificial Sequence
  mutant
MTTTTVSNDQLAKEYVDGVFEQLKNQNSHQAEFLQAAEEIFISLVPVFAQHPEYIKANILSRIVEPDRIISFRVAWQDDNNQVQVNRGYRVQYSNVMGPYKGGLRFHPSVNESIIKFLGFEQIFKNALTGQPVGGGKGGSNFNPKGKSDSEIMRFCQAFMTELYRHIGPDVDGPGGDIGVGAREVGYLWGQYKRITKANESGVLTGKTPGYGGSLARKEATGYGTVYFVEEMLKEVNDSFEDKTVVVSGSGNVSTYAIEKAQAYGAKVVACSDSSGYIYDAEGLDLDVIKEIKEVKGDRISTYVDYRPNATFTEGCTGIWSIPCDIALPCATQNEINGDAARTLISNGVKAIGEGANMPSDLEAINEFLNAGVLFGPAKAANAGGVAVSALEMAQDSSRVFWTFEEVDAKLHQIMKNIYADSKAAADKYGYPGNLVVGANIAGFIKVADGMLAEGIY

SEQ ID NO: 19 - protein, 457 aa, Artificial Sequence
  mutant
MTTTTVSNDQLAKEYVDGVFEQLKNQNSHQAEFLQAAEEIFISLVPVFAQHPEYIKANILSRIVEPDRIISFRVAWQDDNNQVQVNRGYRVQYSNVMGPYKGGLRFHPSVNESIIKFLGFEQIFKNALTGQPVGGGKGGSNFNPKGKSDSEIMRFCQAFMTELYRHIGPDVDVPGGDIGVGRREVGYLWGQYKRITKANESGVLTGKTPGYGGSLARKEATGYGTVYFVEEMLKEVNDSFEDKTVVVSGSGNVSTYAIEKAQAYGAKVVACSDSSGYIYDAEGLDLDVIKEIKEVKGDRISTYVDYRPNATFTEGCTGIWSIPCDIALPCATQNEINGDAARTLISNGVKAIGEGANMPSDLEAINEFLNAGVLFGPAKAANAGGVAVSALEMAQDSSRVFWTFEEVDAKLHQIMKNIYADSKAAADKYGYPGNLVVGANIAGFIKVADGMLAEGIY

SEQ ID NO: 20 - protein, 457 aa, Artificial Sequence
  mutant
MTTTTVSNDQLAKEYVDGVFEQLKNQNSHQAEFLQAAEEIFISLVPVFAQHPEYIKANILSRIVEPDRIISFRVAWQDDNNQVQVNRGYRVQYSNVMGPYKGGLRFHPSVNESIIKFLGFEQIFKNALTGQPIGGGKGGSNFNPKGKSDSEIMRFCQAFMTELYRHIGPDVDSPGGDIGVGRREVGYLWGQYKRITKANESGVLTGKTPGYGGSLARKEATGYGTVYFVEEMLKEVNDSFEDKTVVVSGSGNVSTYAIEKAQAYGAKVVACSDSSGYIYDAEGLDLDVIKEIKEVKGDRISTYVDYRPNATFTEGCTGIWSIPCDIALPCATQNEINGDAARTLISNGVKAIGEGANMPSDLEAINEFLNAGVLFGPAKAANAGGVAVSALEMAQDSSRVFWTFEEVDAKLHQIMKNIYADSKAAADKYGYPGNLVVGANIAGFIKVADGMLAEGIY

SEQ ID NO: 21 - protein, 457 aa, Artificial Sequence; identical to SEQ ID NO: 8
  mutant

SEQ ID NO: 22 - protein, 457 aa, Artificial Sequence
  mutant
MTTTTVSNDQLAKEYVDGVFEQLKNQNSHQAEFLQAAEEIFISLVPVFAQHPEYIKANILSRIVEPDRIISFRVAWQDDNNQVQVNRGYRVQYSNVMGPYKGGLRFHPSVNESIIKFLGFEQIFKNALTGQLVGGGKGGSNFNPKGKSDSEIMRFCQAFMTELYRHIGPDVDSPGGDIGVGAREVGYLWGQYKRITKANESGVLTGKTPGYGGSLARKEATGYGTVYFVEEMLKEVNDSFEDKTVVVSGSGNVSTYAIEKAQAYGAKVVACSDSSGYIYDAEGLDLDVIKEIKEVKGDRISTYVDYRPNATFTEGCTGIWSIPCDIALPCATQNEINGDAARTLISNGVKAIGEGANMPSDLEAINEFLNAGVLFGPAKAANAGGVAVSALEMAQDSSRVFWTFEEVDAKLHQIMKNIYADSKAAADKYGYPGNLVVGANIAGFIKVADGMLAEGIY

SEQ ID NO: 23 - protein, 457 aa, Artificial Sequence
  mutant
MTTTTVSNDQLAKEYVDGVFEQLKNQNSHQAEFLQAAEEIFISLVPVFAQHPEYIKANILSRIVEPDRIISFRVAWQDDNNQVQVNRGYRVQYSNVMGPYKGGLRFHPSVNESIIKFLGFEQIFKNALTGQLVGGGKGGSNFNPKGKSDSEIMRFCQAFMTELYRHIGPDVDGPGGDIGVGAREVGYLWGQYKRITKANESGVLTGKTPGYGGSLARKEATGYGTVYFVEEMLKEVNDSFEDKTVVVSGSGNVSTYAIEKAQAYGAKVVACSDSSGYIYDAEGLDLDVIKEIKEVKGDRISTYVDYRPNATFTEGCTGIWSIPCDIALPCATQNEINGDAARTLISNGVKAIGEGANMPSDLEAINEFLNAGVLFGPAKAANAGGVAVSALEMAQDSSRVFWTFEEVDAKLHQIMKNIYADSKAAADKYGYPGNLVVGANIAGFIKVADGMLAEGIY

SEQ ID NO: 24 - protein, 457 aa, Artificial Sequence
  mutant
MTTTTVSNDQLAKEYVDGVFEQLKNQNSHQAEFLQAAEEIFISLVPVFAQHPEYIKANILSRIVEPDRIISFRVAWQDDNNQVQVNRGYRVQYSNVMGPYKGGLRFHPSVNESIIKFLGFEQIFKNALTGQLVGGGKGGSNFNPKGKSDSEIMRFCQAFMTELYRHIGPDVDVPGGDIGVGRREVGYLWGQYKRITKANESGVLTGKTPGYGGSLARKEATGYGTVYFVEEMLKEVNDSFEDKTVVVSGSGNVSTYAIEKAQAYGAKVVACSDSSGYIYDAEGLDLDVIKEIKEVKGDRISTYVDYRPNATFTEGCTGIWSIPCDIALPCATQNEINGDAARTLISNGVKAIGEGANMPSDLEAINEFLNAGVLFGPAKAANAGGVAVSALEMAQDSSRVFWTFEEVDAKLHQIMKNIYADSKAAADKYGYPGNLVVGANIAGFIKVADGMLAEGIY

SEQ ID NO: 25 - protein, 457 aa, Artificial Sequence
  mutant
MTTTTVSNDQLAKEYVDGVFEQLKNQNSHQAEFLQAAEEIFISLVPVFAQHPEYIKANILSRIVEPDRIISFRVAWQDDNNQVQVNRGYRVQYSNVMGPYKGGLRFHPSVNESIIKFLGFEQIFKNALTGQLIGGGKGGSNFNPKGKSDSEIMRFCQAFMTELYRHIGPDVDSPGGDIGVGRREVGYLWGQYKRITKANESGVLTGKTPGYGGSLARKEATGYGTVYFVEEMLKEVNDSFEDKTVVVSGSGNVSTYAIEKAQAYGAKVVACSDSSGYIYDAEGLDLDVIKEIKEVKGDRISTYVDYRPNATFTEGCTGIWSIPCDIALPCATQNEINGDAARTLISNGVKAIGEGANMPSDLEAINEFLNAGVLFGPAKAANAGGVAVSALEMAQDSSRVFWTFEEVDAKLHQIMKNIYADSKAAADKYGYPGNLVVGANIAGFIKVADGMLAEGIY

SEQ ID NO: 26 - protein, 457 aa, Artificial Sequence
  mutant
MTTTTVSNDQLAKEYVDGVFEQLKNQNSHQAEFLQAAEEIFISLVPVFAQHPEYIKANILSRIVEPDRIISFRVAWQDDNNQVQVNRGYRVQYSNVMGPYKGGLRFHPSVNESIIKFLGFEQIFKNALTGQLIGGGKGGSNFNPKGKSDSEIMRFCQAFMTELYRHIGPDVDGPGGDIGVGRREVGYLWGQYKRITKANESGVLTGKTPGYGGSLARKEATGYGTVYFVEEMLKEVNDSFEDKTVVVSGSGNVSTYAIEKAQAYGAKVVACSDSSGYIYDAEGLDLDVIKEIKEVKGDRISTYVDYRPNATFTEGCTGIWSIPCDIALPCATQNEINGDAARTLISNGVKAIGEGANMPSDLEAINEFLNAGVLFGPAKAANAGGVAVSALEMAQDSSRVFWTFEEVDAKLHQIMKNIYADSKAAADKYGYPGNLVVGANIAGFIKVADGMLAEGIY

SEQ ID NO: 27 - protein, 457 aa, Artificial Sequence
  mutant
MTTTTVSNDQLAKEYVDGVFEQLKNQNSHQAEFLQAAEEIFISLVPVFAQHPEYIKANILSRIVEPDRIISFRVAWQDDNNQVQVNRGYRVQYSNVMGPYKGGLRFHPSVNESIIKFLGFEQIFKNALTGQPVGGGKGGSNFNPKGKSDSEIMRFCQAFMTELYRHIGPDVDSPGGDIGVGRREVGYLWGQYKRITKANESGVLTGKTPGYGGSLARKEATGYGTVYFVEEMLKEVNDSFEDKTVVVSGSGNVSTYAIEKAQAYGAKVVACSDSSGYIYDAEGLDLDVIKEIKEVKGDRISTYVDYRPNATFTEGCTGIWSIPCDIALPCATQNEINGDAARTLISNGVKAIGEGANMPSDLEAINEFLNAGVLFGPAKAANAGGVAVSALEMAQDSSRVFWTFEEVDAKLHQIMKNIYADSKAAADKYGYPGNLVVGANIAGFIKVADGMLAEGIY

SEQ ID NO: 28 - protein, 457 aa, Artificial Sequence
  mutant
MTTTTVSNDQLAKEYVDGVFEQLKNQNSHQAEFLQAAEEIFISLVPVFAQHPEYIKANILSRIVEPDRIISFRVAWQDDNNQVQVNRGYRVQYSNVMGPYKGGLRFHPSVNESIIKFLGFEQIFKNALTGQPVGGGKGGSNFNPKGKSDSEIMRFCQAFMTELYRHIGPDVDGPGGDIGVGRREVGYLWGQYKRITKANESGVLTGKTPGYGGSLARKEATGYGTVYFVEEMLKEVNDSFEDKTVVVSGSGNVSTYAIEKAQAYGAKVVACSDSSGYIYDAEGLDLDVIKEIKEVKGDRISTYVDYRPNATFTEGCTGIWSIPCDIALPCATQNEINGDAARTLISNGVKAIGEGANMPSDLEAINEFLNAGVLFGPAKAANAGGVAVSALEMAQDSSRVFWTFEEVDAKLHQIMKNIYADSKAAADKYGYPGNLVVGANIAGFIKVADGMLAEGIY

SEQ ID NO: 29 - protein, 457 aa, Artificial Sequence
  mutant
MTTTTVSNDQLAKEYVDGVFEQLKNQNSHQAEFLQAAEEIFISLVPVFAQHPEYIKANILSRIVEPDRIISFRVAWQDDNNQVQVNRGYRVQYSNVMGPYKGGLRFHPSVNESIIKFLGFEQIFKNALTGQLVGGGKGGSNFNPKGKSDSEIMRFCQAFMTELYRHIGPDVDSPGGDIGVGRREVGYLWGQYKRITKANESGVLTGKTPGYGGSLARKEATGYGTVYFVEEMLKEVNDSFEDKTVVVSGSGNVSTYAIEKAQAYGAKVVACSDSSGYIYDAEGLDLDVIKEIKEVKGDRISTYVDYRPNATFTEGCTGIWSIPCDIALPCATQNEINGDAARTLISNGVKAIGEGANMPSDLEAINEFLNAGVLFGPAKAANAGGVAVSALEMAQDSSRVFWTFEEVDAKLHQIMKNIYADSKAAADKYGYPGNLVVGANIAGFIKVADGMLAEGIY

SEQ ID NO: 30 - protein, 457 aa, Artificial Sequence
  mutant
MTTTTVSNDQLAKEYVDGVFEQLKNQNSHQAEFLQAAEEIFISLVPVFAQHPEYIKANILSRIVEPDRIISFRVAWQDDNNQVQVNRGYRVQYSNVMGPYKGGLRFHPSVNESIIKFLGFEQIFKNALTGQLVGGGKGGSNFNPKGKSDSEIMRFCQAFMTELYRHIGPDVDGPGGDIGVGRREVGYLWGQYKRITKANESGVLTGKTPGYGGSLARKEATGYGTVYFVEEMLKEVNDSFEDKTVVVSGSGNVSTYAIEKAQAYGAKVVACSDSSGYIYDAEGLDLDVIKEIKEVKGDRISTYVDYRPNATFTEGCTGIWSIPCDIALPCATQNEINGDAARTLISNGVKAIGEGANMPSDLEAINEFLNAGVLFGPAKAANAGGVAVSALEMAQDSSRVFWTFEEVDAKLHQIMKNIYADSKAAADKYGYPGNLVVGANIAGFIKVADGMLAEGIY

SEQ ID NO: 31 - protein, 457 aa, Artificial Sequence
  mutant
MTITTVSNEQLAKEYVDGVFEQLKQQNCHQAEFLQAAEEIFISLVPVFVQHPEYIKANILSRIVEPDRIISFRVAWQDDHNQVQVNRGYRVQYSNVMGPYKGGLRFHPSVNESIIKFLGFEQIFKNALTGQPIGGGKGGSNFDPKGKSDSEIMRFCQAFMTELYRHIGPDVDVPGGDIGVGAREVGYLWGQYKRLTKASESGVLTGKTPGYGGSLARKEATGYGTVYFVNEMLKDVNDSFEGKTVVVSGSGNVSTYAIEKAQQYGAKVVACSDSSGYIYDPEGLDLDVIKEIKEVKGDRISTYVSYRPNATFTNGCTGIWTIPCDIALPCATQNEINGESARTLISNGVKAIGEGANMPSDLEAINEFLNAGVLFGPAKAANAGGVAVSALEMAQDSSRVFWSFEEVDAKLHQIMKDIYSDSKAAAEKYGFPGNLVMGANIAGFIKVADGMLTEGIY

SEQ ID NO: 32 - protein, 457 aa, Artificial Sequence
  mutant
MTITTVSNEQLAKEYVDGVFEQLKQQNCHQAEFLQAAEEIFISLVPVFVQHPEYIKANILSRIVEPDRIISFRVAWQDDHNQVQVNRGYRVQYSNVMGPYKGGLRFHPSVNESIIKFLGFEQIFKNALTGQLIGGGKGGSNFDPKGKSDSEIMRFCQAFMTELYRHIGPDVDVPGGDIGVGAREVGYLWGQYKRLTKASESGVLTGKTPGYGGSLARKEATGYGTVYFVNEMLKDVNDSFEGKTVVVSGSGNVSTYAIEKAQQYGAKVVACSDSSGYIYDPEGLDLDVIKEIKEVKGDRISTYVSYRPNATFTNGCTGIWTIPCDIALPCATQNEINGESARTLISNGVKAIGEGANMPSDLEAINEFLNAGVLFGPAKAANAGGVAVSALEMAQDSSRVFWSFEEVDAKLHQIMKDIYSDSKAAAEKYGFPGNLVMGANIAGFIKVADGMLTEGIY

SEQ ID NO: 33 - protein, 457 aa, Artificial Sequence; identical to SEQ ID NO: 32
  mutant

SEQ ID NO: 34 - protein, 457 aa, Artificial Sequence
  mutant
MTITTVSNEQLAKEYVDGVFEQLKQQNCHQAEFLQAAEEIFISLVPVFVQHPEYIKANILSRIVEPDRIISFRVAWQDDHNQVQVNRGYRVQYSNVMGPYKGGLRFHPSVNESIIKFLGFEQIFKNALTGQPIGGGKGGSNFDPKGKSDSEIMRFCQAFMTELYRHIGPDVDSPGGDIGVGAREVGYLWGQYKRLTKASESGVLTGKTPGYGGSLARKEATGYGTVYFVNEMLKDVNDSFEGKTVVVSGSGNVSTYAIEKAQQYGAKVVACSDSSGYIYDPEGLDLDVIKEIKEVKGDRISTYVSYRPNATFTNGCTGIWTIPCDIALPCATQNEINGESARTLISNGVKAIGEGANMPSDLEAINEFLNAGVLFGPAKAANAGGVAVSALEMAQDSSRVFWSFEEVDAKLHQIMKDIYSDSKAAAEKYGFPGNLVMGANIAGFIKVADGMLTEGIY

SEQ ID NO: 35 - protein, 457 aa, Artificial Sequence
  mutant
MTITTVSNEQLAKEYVDGVFEQLKQQNCHQAEFLQAAEEIFISLVPVFVQHPEYIKANILSRIVEPDRIISFRVAWQDDHNQVQVNRGYRVQYSNVMGPYKGGLRFHPSVNESIIKFLGFEQIFKNALTGQPIGGGKGGSNFDPKGKSDSEIMRFCQAFMTELYRHIGPDVDGPGGDIGVGAREVGYLWGQYKRLTKASESGVLTGKTPGYGGSLARKEATGYGTVYFVNEMLKDVNDSFEGKTVVVSGSGNVSTYAIEKAQQYGAKVVACSDSSGYIYDPEGLDLDVIKEIKEVKGDRISTYVSYRPNATFTNGCTGIWTIPCDIALPCATQNEINGESARTLISNGVKAIGEGANMPSDLEAINEFLNAGVLFGPAKAANAGGVAVSALEMAQDSSRVFWSFEEVDAKLHQIMKDIYSDSKAAAEKYGFPGNLVMGANIAGFIKVADGMLTEGIY

SEQ ID NO: 36 - protein, 457 aa, Artificial Sequence
  mutant
MTITTVSNEQLAKEYVDGVFEQLKQQNCHQAEFLQAAEEIFISLVPVFVQHPEYIKANILSRIVEPDRIISFRVAWQDDHNQVQVNRGYRVQYSNVMGPYKGGLRFHPSVNESIIKFLGFEQIFKNALTGQPIGGGKGGSNFDPKGKSDSEIMRFCQAFMTELYRHIGPDVDVPGGDIGVGRREVGYLWGQYKRLTKASESGVLTGKTPGYGGSLARKEATGYGTVYFVNEMLKDVNDSFEGKTVVVSGSGNVSTYAIEKAQQYGAKVVACSDSSGYIYDPEGLDLDVIKEIKEVKGDRISTYVSYRPNATFTNGCTGIWTIPCDIALPCATQNEINGESARTLISNGVKAIGEGANMPSDLEAINEFLNAGVLFGPAKAANAGGVAVSALEMAQDSSRVFWSFEEVDAKLHQIMKDIYSDSKAAAEKYGFPGNLVMGANIAGFIKVADGMLTEGIY

SEQ ID NO: 37 - protein, 457 aa, Artificial Sequence
  mutant
MTITTVSNEQLAKEYVDGVFEQLKQQNCHQAEFLQAAEEIFISLVPVFVQHPEYIKANILSRIVEPDRIISFRVAWQDDHNQVQVNRGYRVQYSNVMGPYKGGLRFHPSVNESIIKFLGFEQIFKNALTGQPIGGGKGGSNFDPKGKSDSEIMRFCQAFMTELYRHIGPDVDGPGGDIGVGRREVGYLWGQYKRLTKASESGVLTGKTPGYGGSLARKEATGYGTVYFVNEMLKDVNDSFEGKTVVVSGSGNVSTYAIEKAQQYGAKVVACSDSSGYIYDPEGLDLDVIKEIKEVKGDRISTYVSYRPNATFTNGCTGIWTIPCDIALPCATQNEINGESARTLISNGVKAIGEGANMPSDLEAINEFLNAGVLFGPAKAANAGGVAVSALEMAQDSSRVFWSFEEVDAKLHQIMKDIYSDSKAAAEKYGFPGNLVMGANIAGFIKVADGMLTEGIY

SEQ ID NO: 38 - protein, 457 aa, Artificial Sequence
  mutant
MTITTVSNEQLAKEYVDGVFEQLKQQNCHQAEFLQAAEEIFISLVPVFVQHPEYIKANILSRIVEPDRIISFRVAWQDDHNQVQVNRGYRVQYSNVMGPYKGGLRFHPSVNESIIKFLGFEQVFKNALTGQPIGGGKGGSNFDPKGKSDSEIMRFCQAFMTELYRHIGPDVDSPGGDIGVGRREVGYLWGQYKRLTKASESGVLTGKTPGYGGSLARKEATGYGTVYFVNEMLKDVNDSFEGKTVVVSGSGNVSTYAIEKAQQYGAKVVACSDSSGYIYDPEGLDLDVIKEIKEVKGDRISTYVSYRPNATFTNGCTGIWTIPCDIALPCATQNEINGESARTLISNGVKAIGEGANMPSDLEAINEFLNAGVLFGPAKAANAGGVAVSALEMAQDSSRVFWSFEEVDAKLHQIMKDIYSDSKAAAEKYGFPGNLVMGANIAGFIKVADGMLTEGIY

SEQ ID NO: 39 - protein, 457 aa, Artificial Sequence; identical to SEQ ID NO: 8
  mutant

SEQ ID NO: 40 - protein, 457 aa, Artificial Sequence
  mutant
MTTTTVSNDQLAKEYVDGVFEELKNQNSHQAEFLQAAEEIFISLVPVFAQHPEYIKANILSRIVEPDRIISFRVAWQDDNNQVQVNRGYRVQYSNVMGPYKGGLRFHPSVNESIIKFLGFEQIFKNALTGQPIGGGKGGSNFNPKGKSDSEIMRFCQAFMTELYRHIGPDVDGPGGDIGVGAREVGYLWGQYKRITKANESGVLTGKTPGYGGSLARKEATGYGTVYFVEEMLKEVNDSFEDKTVVVSGSGNVSTYAIEKAQAYGAKVVACSDSSGYIYDAEGLDLDVIKEIKEVKGDRISTYVDYRPNATFTEGCTGIWSIPCDIALPCATQNEINGDAARTLISNGVKAIGEGANMPSDLEAINEFLNAGVLFGPAKAANAGGVAVSALEMAQDSSRVFWTFEEVDAKLHQIMKNIYADSKAAADKYGYPGNLVVGANIAGFIKVADGMLAEGIY

SEQ ID NO: 41 - protein, 457 aa, Artificial Sequence
  mutant
MTTTTVSNDQLAKEYVDGVFEQMKNQNSHQAEFLQAAEEIFISLVPVFAQHPEYIKANILSRIVEPDRIISFRVAWQDDNNQVQVNRGYRVQYSNVMGPYKGGLRFHPSVNESIIKFLGFEQIFKNALTGQPIGGGKGGSNFNPKGKSDSEIMRFCQAFMTELYRHIGPDVDGPGGDIGVGAREVGYLWGQYKRITKANESGVLTGKTPGYGGSLARKEATGYGTVYFVEEMLKEVNDSFEDKTVVVSGSGNVSTYAIEKAQAYGAKVVACSDSSGYIYDAEGLDLDVIKEIKEVKGDRISTYVDYRPNATFTEGCTGIWSIPCDIALPCATQNEINGDAARTLISNGVKAIGEGANMPSDLEAINEFLNAGVLFGPAKAANAGGVAVSALEMAQDSSRVFWTFEEVDAKLHQIMKNIYADSKAAADKYGYPGNLVVGANIAGFIKVADGMLAEGIY

SEQ ID NO: 42 - protein, 457 aa, Artificial Sequence
  mutant
MTTTTVSNDQLAKEYVDGVFEQLKNQNSHQAEFLQAAEEIFISLVPVFAQHPEYIQANILSRIVEPDRIISFRVAWQDDNNQVQVNRGYRVQYSNVMGPYKGGLRFHPSVNESIIKFLGFEQIFKNALTGQPIGGGKGGSNFNPKGKSDSEIMRFCQAFMTELYRHIGPDVDGPGGDIGVGAREVGYLWGQYKRITKANESGVLTGKTPGYGGSLARKEATGYGTVYFVEEMLKEVNDSFEDKTVVVSGSGNVSTYAIEKAQAYGAKVVACSDSSGYIYDAEGLDLDVIKEIKEVKGDRISTYVDYRPNATFTEGCTGIWSIPCDIALPCATQNEINGDAARTLISNGVKAIGEGANMPSDLEAINEFLNAGVLFGPAKAANAGGVAVSALEMAQDSSRVFWTFEEVDAKLHQIMKNIYADSKAAADKYGYPGNLVVGANIAGFIKVADGMLAEGIY

SEQ ID NO: 43 - protein, 457 aa, Artificial Sequence
  mutant
MTTTTVSNSQLAKEYVDGVFEQLKNQNSHQAEFLQAAEEIFISLVPVFAQHPEYIKANILSRIVEPDRIISFRVAWQDDNNQVQVNRGYRVQYSNVMGPYKGGLRFHPSVNESIIKFLGFEQIFKNALTGQPIGGGKGGSNFNPKGKSDSEIMRFCQAFMTELYRHIGPDVDGPGGDIGVGAREVGYLWGQYKRITKANESGVLTGKTPGYGGSLARKEATGYGTVYFVEEMLKEVNDSFEDKTVVVSGSGNVSTYAIEKAQAYGAKVVACSDSSGYIYDAEGLDLDVIKEIKEVKGDRISTYVDYRPNATFTEGCTGIWSIPCDIALPCATQNEINGDAARTLISNGVKAIGEGANMPSDLEAINEFLNAGVLFGPAKAANAGGVAVSALEMAQDSSRVFWTFEEVDAKLHQIMKNIYADSKAAADKYGYPGNLVVGANIAGFIKVADGMLAEGIY

SEQ ID NO: 44 - protein, 457 aa, Artificial Sequence
  mutant
MTTTTVSNLQLAKEYVDGVFEQLKNQNSHQAEFLQAAEEIFISLVPVFAQHPEYIKANILSRIVEPDRIISFRVAWQDDNNQVQVNRGYRVQYSNVMGPYKGGLRFHPSVNESIIKFLGFEQIFKNALTGQPIGGGKGGSNFNPKGKSDSEIMRFCQAFMTELYRHIGPDVDGPGGDIGVGAREVGYLWGQYKRITKANESGVLTGKTPGYGGSLARKEATGYGTVYFVEEMLKEVNDSFEDKTVVVSGSGNVSTYAIEKAQAYGAKVVACSDSSGYIYDAEGLDLDVIKEIKEVKGDRISTYVDYRPNATFTEGCTGIWSIPCDIALPCATQNEINGDAARTLISNGVKAIGEGANMPSDLEAINEFLNAGVLFGPAKAANAGGVAVSALEMAQDSSRVFWTFEEVDAKLHQIMKNIYADSKAAADKYGYPGNLVVGANIAGFIKVADGMLAEGIY

SEQ ID NO: 45 - protein, 457 aa, Artificial Sequence
  mutant
MTTTTVSNYQLAKEYVDGVFEQLKNQNSHQAEFLQAAEEIFISLVPVFAQHPEYIKANILSRIVEPDRIISFRVAWQDDNNQVQVNRGYRVQYSNVMGPYKGGLRFHPSVNESIIKFLGFEQIFKNALTGQPIGGGKGGSNFNPKGKSDSEIMRFCQAFMTELYRHIGPDVDGPGGDIGVGAREVGYLWGQYKRITKANESGVLTGKTPGYGGSLARKEATGYGTVYFVEEMLKEVNDSFEDKTVVVSGSGNVSTYAIEKAQAYGAKVVACSDSSGYIYDAEGLDLDVIKEIKEVKGDRISTYVDYRPNATFTEGCTGIWSIPCDIALPCATQNEINGDAARTLISNGVKAIGEGANMPSDLEAINEFLNAGVLFGPAKAANAGGVAVSALEMAQDSSRVFWTFEEVDAKLHQIMKNIYADSKAAADKYGYPGNLVVGANIAGFIKVADGMLAEGIY

SEQ ID NO: 46 - protein, 457 aa, Artificial Sequence
  mutant
MTTTTVSNDQLAKEYVDGVFEQLKDQNSHQAEFLQAAEEIFISLVPVFAQHPEYIKANILSRIVEPDRIISFRVAWQDDNNQVQVNRGYRVQYSNVMGPYKGGLRFHPSVNESIIKFLGFEQIFKNALTGQPIGGGKGGSNFNPKGKSDSEIMRFCQAFMTELYRHIGPDVDGPGGDIGVGAREVGYLWGQYKRITKANESGVLTGKTPGYGGSLARKEATGYGTVYFVEEMLKEVNDSFEDKTVVVSGSGNVSTYAIEKAQAYGAKVVACSDSSGYIYDAEGLDLDVIKEIKEVKGDRISTYVDYRPNATFTEGCTGIWSIPCDIALPCATQNEINGDAARTLISNGVKAIGEGANMPSDLEAINEFLNAGVLFGPAKAANAGGVAVSALEMAQDSSRVFWTFEEVDAKLHQIMKNIYADSKAAADKYGYPGNLVVGANIAGFIKVADGMLAEGIY

SEQ ID NO: 47 - protein, 457 aa, Artificial Sequence
  mutant
MTTTTVSNDQLAKEYVDGVFEQLKNQNSHQAEFLQAAEEIFISLVPVFAQHPEYIKANILSRIVEPDRIISFRVAWQDDNNQVQVNRGYRVQYSNVMGPYKGGLRFHPSVNESIIKFLGFEQIFKNALTGQPIGGGKGGSNFNPKGKSDSEIMRFCQAFMTELYRHIGPDVDGPGGDIGVGAREVGYLWGQYKRITKAWESGVLTGKTPGYGGSLARKEATGYGTVYFVEEMLKEVNDSFEDKTVVVSGSGNVSTYAIEKAQAYGAKVVACSDSSGYIYDAEGLDLDVIKEIKEVKGDRISTYVDYRPNATFTEGCTGIWSIPCDIALPCATQNEINGDAARTLISNGVKAIGEGANMPSDLEAINEFLNAGVLFGPAKAANAGGVAVSALEMAQDSSRVFWTFEEVDAKLHQIMKNIYADSKAAADKYGYPGNLVVGANIAGFIKVADGMLAEGIY

SEQ ID NO: 48 - protein, 457 aa, Artificial Sequence
  mutant
MTTTTVSNDQLAKEYVDGVFEQLKNQNSHQAEFLQAAEEIFISLVPVFAQHPEYIKANILSRIVEPDRIISFRVAWQDDNNQVQVNRGYRVQYSNVMGPYKGGLRFHPSVNESIIKFLGFEQIFKNALTGQPIGGGKGGSNFNPKGKSDSEIMRFCQAFMTELYRHIGPDVDGPGGDIGVGAREVGYLWGQYKRITKAYESGVLTGKTPGYGGSLARKEATGYGTVYFVEEMLKEVNDSFEDKTVVVSGSGNVSTYAIEKAQAYGAKVVACSDSSGYIYDAEGLDLDVIKEIKEVKGDRISTYVDYRPNATFTEGCTGIWSIPCDIALPCATQNEINGDAARTLISNGVKAIGEGANMPSDLEAINEFLNAGVLFGPAKAANAGGVAVSALEMAQDSSRVFWTFEEVDAKLHQIMKNIYADSKAAADKYGYPGNLVVGANIAGFIKVADGMLAEGIY

SEQ ID NO: 49 - protein, 457 aa, Artificial Sequence
  mutant
MTTTTVSNDQLAKEYVDGVFEQLKNQNSHQAEFLQAAEEIFISLVPVFAQHPEYIKANILSRIVEPDRIISFRVAWQDDNNQVQVNRGYRVQYSNVMGPYKGGLRFHPSVNESIIKFLGFEQIFKNALTGQPIGGGKGGSNFNPKGKSDSEIMRFCQAFMTELYRHIGPDVDGPGGDIGVGAREVGYLWGQYKRITKANESGVLTGKTPGYGGSLARKEATGYGTVYFVEEMLKEVNDSFEGKTVVVSGSGNVSTYAIEKAQAYGAKVVACSDSSGYIYDAEGLDLDVIKEIKEVKGDRISTYVDYRPNATFTEGCTGIWSIPCDIALPCATQNEINGDAARTLISNGVKAIGEGANMPSDLEAINEFLNAGVLFGPAKAANAGGVAVSALEMAQDSSRVFWTFEEVDAKLHQIMKNIYADSKAAADKYGYPGNLVVGANIAGFIKVADGMLAEGIY

SEQ ID NO: 50 - protein, 457 aa, Artificial Sequence
  mutant
MTTTTVSNDQLAKEYVDGVFEQLKNQNSHQAEFLQAAEEIFISLVPVFAQHPEYIKANILSRIVEPDRIISFRVAWQDDNNQVQVNRGYRVQYSNVMGPYKGGLRFHPSVNESIIKFLGFEQIFKNALTGQPIGGGKGGSNFEPKGKSDSEIMRFCQAFMTELYRHIGPDVDGPGGDIGVGAREVGYLWGQYKRITKANESGVLTGKTPGYGGSLARKEATGYGTVYFVEEMLKEVNDSFEDKTVVVSGSGNVSTYAIEKAQAYGAKVVACSDSSGYIYDAEGLDLDVIKEIKEVKGDRISTYVDYRPNATFTEGCTGIWSIPCDIALPCATQNEINGDAARTLISNGVKAIGEGANMPSDLEAINEFLNAGVLFGPAKAANAGGVAVSALEMAQDSSRVFWTFEEVDAKLHQIMKNIYADSKAAADKYGYPGNLVVGANIAGFIKVADGMLAEGIY

SEQ ID NO: 51 - protein, 457 aa, Artificial Sequence
  mutant
MTTTTVSNDQLAKEYVDGVFEQLKNQNSHQAEFLQAAEEIFISLVPVFAQHPEYIKANILSRIVEPDRIISFRVAWQDDNNQVQVNRGYRVQYSNVMGPYKGGLRFHPSVNESIIKFLGFEQIFKNALTGQPIGGGKGGSNFNPKGKSDSEIMRFCQAFMTELYRHIGPDVDGPGGDIGVGAREVGYLWGQYKRITKANESGVLTGKTPGYGGSLARKEATGYGTVYFVEEMLKEVNDSFEDKTVVVSGSGNVSTYAIEKAQSYGAKVVACSDSSGYIYDAEGLDLDVIKEIKEVKGDRISTYVDYRPNATFTEGCTGIWSIPCDIALPCATQNEINGDAARTLISNGVKAIGEGANMPSDLEAINEFLNAGVLFGPAKAANAGGVAVSALEMAQDSSRVFWTFEEVDAKLHQIMKNIYADSKAAADKYGYPGNLVVGANIAGFIKVADGMLAEGIY

SEQ ID NO: 52 - protein, 457 aa, Artificial Sequence
  mutant
MTTTTVSNDQLAKEYVDGVFEQLKNQNSHQAEFLQAAEEIFISLVPVFAQHPEYIKANILSRIVEPDRIISFRVAWQDDNNQVQVNRGYRVQYSNVMGPYKGGLRFHPSVNESIIKFLGFEQIFKNALTGQPIGGGKGGSNFNPKGKSDSEIMRFCQAFMTELYRHIGPDVDGPGGDIGVGAREVGYLWGQYKRITKANESGVLTGKTPGYGGSLARKEATGYGTVYFVEEMLKEVNDSFEDKTVVVSGSGNVSTYAIEKAQKYGAKVVACSDSSGYIYDAEGLDLDVIKEIKEVKGDRISTYVDYRPNATFTEGCTGIWSIPCDIALPCATQNEINGDAARTLISNGVKAIGEGANMPSDLEAINEFLNAGVLFGPAKAANAGGVAVSALEMAQDSSRVFWTFEEVDAKLHQIMKNIYADSKAAADKYGYPGNLVVGANIAGFIKVADGMLAEGIY

SEQ ID NO: 53 - protein, 457 aa, Artificial Sequence
  mutant
MTTTTVSNDQLAKEYVDGVFEQLKNQNSHQAEFLQAAEEIFISLVPVFAQHPEYIKANILSRIVEPDRIISFRVAWQDDNNQVQVNRGYRVQYSNVMGPYKGGLRFHPSVNESIIKFLGFEQIFKNALTGQPIGGGKGGSNFNPKGKSDSEIMRFCQAFMTELYRHIGPDVDGPGGDIGVGAREVGYLWGQYKRITKANESGVLTGKTPGYGGSLARKEATGYGTVYFVEEMLKEVNDSFEDKTVVVSGSGNVSTYAIEKAQAYGAKVVACSDSSGYIYDAEGLDLDVIKEIKEVKGDRISTYVDYRPNATFTEGCTGIWSIPCDIALPCATQNEINGQAARTLISNGVKAIGEGANMPSDLEAINEFLNAGVLFGPAKAANAGGVAVSALEMAQDSSRVFWTFEEVDAKLHQIMKNIYADSKAAADKYGYPGNLVVGANIAGFIKVADGMLAEGIY

SEQ ID NO: 54 - protein, 457 aa, Artificial Sequence
  mutant
MTTTTVSNDQLAKEYVDGVFEQLKNQNSHQAEFLQAAEEIFISLVPVFAQHPEYIKANILSRIVEPDRIISFRVAWQDDNNQVQVNRGYRVQYSNVMGPYKGGLRFHPSVNESIIKFLGFEQIFKNALTGQPIGGGKGGSNFNPKGKSDSEIMRFCQAFMTELYRHIGPDVDGPGGDIGVGAREVGYLWGQYKRITKANESGVLTGKTPGYGGSLARKEATGYGTVYFVEEMLKEVNDSFEDKTVVVSGSGNVSTYAIEKAQAYGAKVVACSDSSGYIYDAEGLDLDVIKEIKEVKGDRISTYVDYRPNATFTEGCTGIWSIPCDIALPCATQNEINGDAARTLISNGVKAIGEGANMPSDLEAINEFLNAGVLFGPAKAANAGGVAVSALEMAQDSSRVFWTFEEVDAKLHQIMKNIYRDSKAAADKYGYPGNLVVGANIAGFIKVADGMLAEGIY

SEQ ID NO: 55 - protein, 457 aa, Artificial Sequence
  mutant
MTTTTVSNDQLAKEYVDGVFEQLKNQNSHQAEFLQAAEEIFISLVPVFAQHPEYIKANILSRIVEPDRIISFRVAWQDDNNQVQVNRGYRVQYSNVMGPYKGGLRFHPSVNESIIKFLGFEQIFKNALTGQPIGGGKGGSNFNPKGKSDSEIMRFCQAFMTELYRHIGPDVDGPGGDIGVGAREVGYLWGQYKRITKANESGVLTGKTPGYGGSLARKEATGYGTVYFVEEMLKEVNDSFEDKTVVVSGSGNVSTYAIEKAQAYGAKVVACSDSSGYIYDAEGLDLDVIKEIKEVKGDRISTYVDYRPNATFTEGCTGIWSIPCDIALPCATQNEINGDAARTLISNGVKAIGEGANMPSDLEAINEFLNAGVLFGPAKAANAGGVAVSALEMAQDSSRVFWTFEEVDAKLHQIMKNIYADSKAAADKYGSPGNLVVGANIAGFIKVADGMLAEGIY

SEQ ID NO: 56 - protein, 457 aa, Artificial Sequence
  mutant
MTTTTVSNDQLAKEYVDGVFEQLKNQNSHQAEFLQAAEEIFISLVPVFAQHPEYIKANILSRIVEPDRIISFRVAWQDDNNQVQVNRGYRVQYSNVMGPYKGGLRFHPSVNESIIKFLGFEQIFKNALTGQPIGGGKGGSNFNPKGKSDSEIMRFCQAFMTELYRHIGPDVDGPGGDIGVGAREVGYLWGQYKRITKANESGVLTGKTPGYGGSLARKEATGYGTVYFVEEMLKEVNDSFEDKTVVVSGSGNVSTYAIEKAQAYGAKVVACSDSSGYIYDAEGLDLDVIKEIKEVKGDRISTYVDYRPNATFTEGCTGIWSIPCDIALPCATQNEINGDAARTLISNGVKAIGEGANMPSDLEAINEFLNAGVLFGPAKAANAGGVAVSALEMAQDSSRVFWTFEEVDAKLHQIMKNIYADSKAAADKYGYPGNLVKGANIAGFIKVADGMLAEGIY

SEQ ID NO: 57 - protein, 457 aa, Artificial Sequence
  mutant
MTTTTVSNDQLAKEYVDGVFEQLKNQNSHQAEFLQAAEEIFISLVPVFAQHPEYIQANILSRIVEPDRIISFRVAWQDDNNQVQVNRGYRVQYSNVMGPYKGGLRFHPSVNESIIKFLGFEQIFKNALTGQPIGGGKGGSNFNPKGKSDSEIMRFCQAFMTELYRHIGPDVDGPGGDIGVGAREVGYLWGQYKRITKAWESGVLTGKTPGYGGSLARKEATGYGTVYFVEEMLKEVNDSFEDKTVVVSGSGNVSTYAIEKAQAYGAKVVACSDSSGYIYDAEGLDLDVIKEIKEVKGDRISTYVDYRPNATFTEGCTGIWSIPCDIALPCATQNEINGDAARTLISNGVKAIGEGANMPSDLEAINEFLNAGVLFGPAKAANAGGVAVSALEMAQDSSRVFWTFEEVDAKLHQIMKNIYADSKAAADKYGYPGNLVVGANIAGFIKVADGMLAEGIY

SEQ ID NO: 58 - protein, 457 aa, Artificial Sequence
  mutant
MTTTTVSNDQLAKEYVDGVFEELKNQNSHQAEFLQAAEEIFISLVPVFAQHPEYIKANILSRIVEPDRIISFRVAWQDDNNQVQVNRGYRVQYSNVMGPYKGGLRFHPSVNESIIKFLGFEQIFKNALTGQPIGGGKGGSNFNPKGKSDSEIMRFCQAFMTELYRHIGPDVDGPGGDIGVGAREVGYLWGQYKRITKAWESGVLTGKTPGYGGSLARKEATGYGTVYFVEEMLKEVNDSFEDKTVVVSGSGNVSTYAIEKAQAYGAKVVACSDSSGYIYDAEGLDLDVIKEIKEVKGDRISTYVDYRPNATFTEGCTGIWSIPCDIALPCATQNEINGDAARTLISNGVKAIGEGANMPSDLEAINEFLNAGVLFGPAKAANAGGVAVSALEMAQDSSRVFWTFEEVDAKLHQIMKNIYADSKAAADKYGYPGNLVVGANIAGFIKVADGMLAEGIY

SEQ ID NO: 59 - protein, 457 aa, Artificial Sequence
  mutant
MTTTTVSNDQLAKEYVDGVFEQLKNQNSHQAEFLQAAEEIFISLVPVFAQHPEYIQANILSRIVEPDRIISFRVAWQDDNNQVQVNRGYRVQYSNVMGPYKGGLRFHPSVNESIIKFLGFEQIFKNALTGQPIGGGKGGSNFNPKGKSDSEIMRFCQAFMTELYRHIGPDVDGPGGDIGVGAREVGYLWGQYKRITKAYESGVLTGKTPGYGGSLARKEATGYGTVYFVEEMLKEVNDSFEDKTVVVSGSGNVSTYAIEKAQAYGAKVVACSDSSGYIYDAEGLDLDVIKEIKEVKGDRISTYVDYRPNATFTEGCTGIWSIPCDIALPCATQNEINGDAARTLISNGVKAIGEGANMPSDLEAINEFLNAGVLFGPAKAANAGGVAVSALEMAQDSSRVFWTFEEVDAKLHQIMKNIYADSKAAADKYGYPGNLVVGANIAGFIKVADGMLAEGIY

SEQ ID NO: 60 - protein, 457 aa, Artificial Sequence
  mutant
MTTTTVSNDQLAKEYVDGVFEELKNQNSHQAEFLQAAEEIFISLVPVFAQHPEYIKANILSRIVEPDRIISFRVAWQDDNNQVQVNRGYRVQYSNVMGPYKGGLRFHPSVNESIIKFLGFEQIFKNALTGQPIGGGKGGSNFNPKGKSDSEIMRFCQAFMTELYRHIGPDVDGPGGDIGVGAREVGYLWGQYKRITKAYESGVLTGKTPGYGGSLARKEATGYGTVYFVEEMLKEVNDSFEDKTVVVSGSGNVSTYAIEKAQAYGAKVVACSDSSGYIYDAEGLDLDVIKEIKEVKGDRISTYVDYRPNATFTEGCTGIWSIPCDIALPCATQNEINGDAARTLISNGVKAIGEGANMPSDLEAINEFLNAGVLFGPAKAANAGGVAVSALEMAQDSSRVFWTFEEVDAKLHQIMKNIYADSKAAADKYGYPGNLVVGANIAGFIKVADGMLAEGIY

SEQ ID NO: 61 - protein, 457 aa, Artificial Sequence
  mutant
MTTTTVSNDQLAKEYVDGVFEQLKNQNSHQAEFLQAAEEIFISLVPVFAQHPEYIQANILSRIVEPDRIISFRVAWQDDNNQVQVNRGYRVQYSNVMGPYKGGLRFHPSVNESIIKFLGFEQIFKNALTGQPIGGGKGGSNFNPKGKSDSEIMRFCQAFMTELYRHIGPDVDGPGGDIGVGAREVGYLWGQYKRITKAYESGVLTGKTPGYGGSLARKEATGYGTVYFVEEMLKEVNDSFEDKTVVVSGSGNVSTYAIEKAQAYGAKVVACSDSSGYIYDAEGLDLDVIKEIKEVKGDRISTYVDYRPNATFTEGCTGIWSIPCDIALPCATQNEINGDAARTLISNGVKAIGEGANMPSDLEAINEFLNAGVLFGPAKAANAGGVAVSALEMAQDSSRVFWTFEEVDAKLHQIMKNIYRDSKAAADKYGYPGNLVVGANIAGFIKVADGMLAEGIY

SEQ ID NO: 62 - protein, 457 aa, Artificial Sequence
  mutant
MTTTTVSNDQLAKEYVDGVFEELKNQNSHQAEFLQAAEEIFISLVPVFAQHPEYIKANILSRIVEPDRIISFRVAWQDDNNQVQVNRGYRVQYSNVMGPYKGGLRFHPSVNESIIKFLGFEQIFKNALTGQPIGGGKGGSNFNPKGKSDSEIMRFCQAFMTELYRHIGPDVDGPGGDIGVGAREVGYLWGQYKRITKAYESGVLTGKTPGYGGSLARKEATGYGTVYFVEEMLKEVNDSFEDKTVVVSGSGNVSTYAIEKAQAYGAKVVACSDSSGYIYDAEGLDLDVIKEIKEVKGDRISTYVDYRPNATFTEGCTGIWSIPCDIALPCATQNEINGDAARTLISNGVKAIGEGANMPSDLEAINEFLNAGVLFGPAKAANAGGVAVSALEMAQDSSRVFWTFEEVDAKLHQIMKNIYRDSKAAADKYGYPGNLVVGANIAGFIKVADGMLAEGIY

SEQ ID NO: 63 - protein, 457 aa, Artificial Sequence
  mutant
MTTTTVSNDQLAKEYVDGVFEELKNQNSHQAEFLQAAEEIFISLVPVFAQHPEYIQANILSRIVEPDRIISFRVAWQDDNNQVQVNRGYRVQYSNVMGPYKGGLRFHPSVNESIIKFLGFEQIFKNALTGQPIGGGKGGSNFNPKGKSDSEIMRFCQAFMTELYRHIGPDVDGPGGDIGVGAREVGYLWGQYKRITKAYESGVLTGKTPGYGGSLARKEATGYGTVYFVEEMLKEVNDSFEDKTVVVSGSGNVSTYAIEKAQAYGAKVVACSDSSGYIYDAEGLDLDVIKEIKEVKGDRISTYVDYRPNATFTEGCTGIWSIPCDIALPCATQNEINGDAARTLISNGVKAIGEGANMPSDLEAINEFLNAGVLFGPAKAANAGGVAVSALEMAQDSSRVFWTFEEVDAKLHQIMKNIYADSKAAADKYGYPGNLVVGANIAGFIKVADGMLAEGIY

SEQ ID NO: 64 - protein, 457 aa, Artificial Sequence
  mutant
MTTTTVSNDQLAKEYVDGVFEELKNQNSHQAEFLQAAEEIFISLVPVFAQHPEYIQANILSRIVEPDRIISFRVAWQDDNNQVQVNRGYRVQYSNVMGPYKGGLRFHPSVNESIIKFLGFEQIFKNALTGQPIGGGKGGSNFNPKGKSDSEIMRFCQAFMTELYRHIGPDVDGPGGDIGVGAREVGYLWGQYKRITKAWESGVLTGKTPGYGGSLARKEATGYGTVYFVEEMLKEVNDSFEDKTVVVSGSGNVSTYAIEKAQAYGAKVVACSDSSGYIYDAEGLDLDVIKEIKEVKGDRISTYVDYRPNATFTEGCTGIWSIPCDIALPCATQNEINGDAARTLISNGVKAIGEGANMPSDLEAINEFLNAGVLFGPAKAANAGGVAVSALEMAQDSSRVFWTFEEVDAKLHQIMKNIYADSKAAADKYGYPGNLVVGANIAGFIKVADGMLAEGIY

SEQ ID NO: 65 - protein, 457 aa, Artificial Sequence
  mutant
MTTTTVSNDQLAKEYVDGVFEELKNQNSHQAEFLQAAEEIFISLVPVFAQHPEYIQANILSRIVEPDRIISFRVAWQDDNNQVQVNRGYRVQYSNVMGPYKGGLRFHPSVNESIIKFLGFEQIFKNALTGQPIGGGKGGSNFNPKGKSDSEIMRFCQAFMTELYRHIGPDVDGPGGDIGVGAREVGYLWGQYKRITKAYESGVLTGKTPGYGGSLARKEATGYGTVYFVEEMLKEVNDSFEDKTVVVSGSGNVSTYAIEKAQAYGAKVVACSDSSGYIYDAEGLDLDVIKEIKEVKGDRISTYVDYRPNATFTEGCTGIWSIPCDIALPCATQNEINGDAARTLISNGVKAIGEGANMPSDLEAINEFLNAGVLFGPAKAANAGGVAVSALEMAQDSSRVFWTFEEVDAKLHQIMKNIYRDSKAAADKYGYPGNLVVGANIAGFIKVADGMLAEGIY

SEQ ID NO: 66 - protein, 457 aa, Artificial Sequence
  mutant
MTTTTVSNDQLAKEYVDGVFEELKNQNSHQHEFLQAAEEIFISLVPVFAQHPEYIQANILSRIVEPDRIISFRVAWQDDNNQVQVNRGYRVQYSNVMGPYKGGLRFHPSVNESIIKFLGFEQIFKNALTGQPIGGGKGGSNFNPKGKSDSEIMRFCQAFMTELYRHIGPDVDGPGGDIGVGAREVGYLWGQYKRITKAYESGVLTGKTPGYGGSLARKEATGYGTVYFVEEMLKEVNDSFEDKTVVVSGSGNVSTYAIEKAQAYGAKVVACSDSSGYIYDAEGLDLDVIKEIKEVKGDRISTYVDYRPNATFTEGCTGIWSIPCDIALPCATQNEINGDAARTLISNGVKAIGEGANMPSDLEAINEFLNAGVLFGPAKAANAGGVAVSALEMAQDSSRVFWTFEEVDAKLHQIMKNIYRDSKAAADKYGYPGNLVVGANIAGFIKVADGMLAEGIY

SEQ ID NO: 67 - protein, 457 aa, Artificial Sequence
  mutant
MTTTTVSNDQLAKEYVDGVFEELKNQNSHQAEFLQAAEEIFISLVPVFAQHPEYIQANILSRIVEPDRIISFRVAWQDDNNQVQVNRGYRVQYSNVMGPYKGGLRFHPSVNESIIKFLGFEQILKNALTGQPIGGGKGGSNFNPKGKSDSEIMRFCQAFMTELYRHIGPDVDGPGGDIGVGAREVGYLWGQYKRITKAYESGVLTGKTPGYGGSLARKEATGYGTVYFVEEMLKEVNDSFEDKTVVVSGSGNVSTYAIEKAQAYGAKVVACSDSSGYIYDAEGLDLDVIKEIKEVKGDRISTYVDYRPNATFTEGCTGIWSIPCDIALPCATQNEINGDAARTLISNGVKAIGEGANMPSDLEAINEFLNAGVLFGPAKAANAGGVAVSALEMAQDSSRVFWTFEEVDAKLHQIMKNIYRDSKAAADKYGYPGNLVVGANIAGFIKVADGMLAEGIY

SEQ ID NO: 68 - protein, 457 aa, Artificial Sequence
  mutant
MTTTTVSNDQLAKEYVDGVFEELKNQNSHQAEFLQAAEEIFISLVPVFAQHPEYIQANILSRIVEPDRIISFRVAWQDDNNQVQVNRGYRVQYSNVMGPYKGGLRFHPSVNESIIKFLGFEQIFKNALTGQPIGGGKGGSNFNPKGKSDSEIMRFCQAFMTELYRHIGPDVDGPGGDIGVGAREVGYLWGQYKRITKAYESGVLTGKTPGYGGSLGRKEATGYGTVYFVEEMLKEVNDSFEDKTVVVSGSGNVSTYAIEKAQAYGAKVVACSDSSGYIYDAEGLDLDVIKEIKEVKGDRISTYVDYRPNATFTEGCTGIWSIPCDIALPCATQNEINGDAARTLISNGVKAIGEGANMPSDLEAINEFLNAGVLFGPAKAANAGGVAVSALEMAQDSSRVFWTFEEVDAKLHQIMKNIYRDSKAAADKYGYPGNLVVGANIAGFIKVADGMLAEGIY

SEQ ID NO: 69 - protein, 457 aa, Artificial Sequence
  mutant
MTTTTVSNDQLAKEYVDGVFEELKNQNSHQHEFLQAAEEIFISLVPVFAQHPEYIQANILSRIVEPDRIISFRVAWQDDNNQVQVNRGYRVQYSNVMGPYKGGLRFHPSVNESIIKFLGFEQILKNALTGQPIGGGKGGSNFNPKGKSDSEIMRFCQAFMTELYRHIGPDVDGPGGDIGVGAREVGYLWGQYKRITKAYESGVLTGKTPGYGGSLARKEATGYGTVYFVEEMLKEVNDSFEDKTVVVSGSGNVSTYAIEKAQAYGAKVVACSDSSGYIYDAEGLDLDVIKEIKEVKGDRISTYVDYRPNATFTEGCTGIWSIPCDIALPCATQNEINGDAARTLISNGVKAIGEGANMPSDLEAINEFLNAGVLFGPAKAANAGGVAVSALEMAQDSSRVFWTFEEVDAKLHQIMKNIYRDSKAAADKYGYPGNLVVGANIAGFIKVADGMLAEGIY

SEQ ID NO: 70 - protein, 457 aa, Artificial Sequence
  mutant
MTTTTVSNDQLAKEYVDGVFEELKNQNSHQHEFLQAAEEIFISLVPVFAQHPEYIQANILSRIVEPDRIISFRVAWQDDNNQVQVNRGYRVQYSNVMGPYKGGLRFHPSVNESIIKFLGFEQIFKNALTGQPIGGGKGGSNFNPKGKSDSEIMRFCQAFMTELYRHIGPDVDGPGGDIGVGAREVGYLWGQYKRITKAYESGVLTGKTPGYGGSLGRKEATGYGTVYFVEEMLKEVNDSFEDKTVVVSGSGNVSTYAIEKAQAYGAKVVACSDSSGYIYDAEGLDLDVIKEIKEVKGDRISTYVDYRPNATFTEGCTGIWSIPCDIALPCATQNEINGDAARTLISNGVKAIGEGANMPSDLEAINEFLNAGVLFGPAKAANAGGVAVSALEMAQDSSRVFWTFEEVDAKLHQIMKNIYRDSKAAADKYGYPGNLVVGANIAGFIKVADGMLAEGIY

SEQ ID NO: 71 - protein, 457 aa, Artificial Sequence
  mutant
MTTTTVSNDQLAKEYVDGVFEELKNQNSHQAEFLQAAEEIFISLVPVFAQHPEYIQANILSRIVEPDRIISFRVAWQDDNNQVQVNRGYRVQYSNVMGPYKGGLRFHPSVNESIIKFLGFEQILKNALTGQPIGGGKGGSNFNPKGKSDSEIMRFCQAFMTELYRHIGPDVDGPGGDIGVGAREVGYLWGQYKRITKAYESGVLTGKTPGYGGSLGRKEATGYGTVYFVEEMLKEVNDSFEDKTVVVSGSGNVSTYAIEKAQAYGAKVVACSDSSGYIYDAEGLDLDVIKEIKEVKGDRISTYVDYRPNATFTEGCTGIWSIPCDIALPCATQNEINGDAARTLISNGVKAIGEGANMPSDLEAINEFLNAGVLFGPAKAANAGGVAVSALEMAQDSSRVFWTFEEVDAKLHQIMKNIYRDSKAAADKYGYPGNLVVGANIAGFIKVADGMLAEGIY

SEQ ID NO: 72 - protein, 457 aa, Artificial Sequence
  mutant
MTTTTVSNDQLAKEYVDGVFEELKNQNSHQHEFLQAAEEIFISLVPVFAQHPEYIQANILSRIVEPDRIISFRVAWQDDNNQVQVNRGYRVQYSNVMGPYKGGLRFHPSVNESIIKFLGFEQILKNALTGQPIGGGKGGSNFNPKGKSDSEIMRFCQAFMTELYRHIGPDVDGPGGDIGVGAREVGYLWGQYKRITKAYESGVLTGKTPGYGGSLGRKEATGYGTVYFVEEMLKEVNDSFEDKTVVVSGSGNVSTYAIEKAQAYGAKVVACSDSSGYIYDAEGLDLDVIKEIKEVKGDRISTYVDYRPNATFTEGCTGIWSIPCDIALPCATQNEINGDAARTLISNGVKAIGEGANMPSDLEAINEFLNAGVLFGPAKAANAGGVAVSALEMAQDSSRVFWTFEEVDAKLHQIMKNIYRDSKAAADKYGYPGNLVVGANIAGFIKVADGMLAEGIY